European Patent Specification EP 4 448 548 B1, published October 22, 2025. Title: BACTERIOPHAGE LAMBDA-VACCINE SYSTEM. Applicant: The United States of America, as represented by the Secretary, Department of Health and Human Services. The sequence listing filed with the application follows.

SEQUENCE LISTING (69 sequences)

SEQ ID NO: 1 - protein, 110 aa, bacteriophage lambda
MTSKETFTHYQPQGNSDPAHTATAPGGLSAKAPAMTPLMLDTSSRKLVAWDGTTDGAAVGILAVAADQTSTTLTFYKSGTFRYEDVLWPEAASDETKKRTAFAGTAISIV

SEQ ID NO: 2 - protein, 5 aa, synthetic construct
GGGGS

SEQ ID NO: 3 - protein, 341 aa, bacteriophage lambda
MSMYTTAQLLAANEQKFKFDPLFLRLFFRESYPFTTEKVYLSQIPGLVNMALYVSPIVSGEVIRSRGGSTSEFTPGYVKPKHEVNPQMTLRRLPDEDPQNLADPAYRRRRIIMQNMRDEELAIAQVEEMQAVSAVLKGKYTMTGEAFDPVEVDMGRSEENNITQSGGTEWSKRDKSTYDPTDDIEAYALNASGVVNIIVFDPKGWALFRSFKAVKEKLDTRRGSNSELETAVKDLGKAVSYKGMYGDVAIVVYSGQYVENGVKKNFLPDNTMVLGNTQARGLRTYGCIQDADAQREGINASARYPKNWVTTGDPAREFTMIQSAPLMLLADPDEFVSVQLA

SEQ ID NO: 4 - protein, 133 aa, Severe acute respiratory syndrome-related coronavirus
KRVDFCGKGYHLMSFPQSAPHGVVFLHVTYVPAQEKNFTTAPAICHDGKAHFPREGVFVSNGTHWFVTQRNFYEPQIITTDNTFVSGNCDVVIGIVNNTVYDPLQPELDSFKEELDKYFKNHTSPDVDLGDIS

SEQ ID NO: 5 - protein, 143 aa, Plasmodium sp.
ASKSKEHKSKGKKDKGKKDKGKHKKAKKEKVKKHVVKNVIEDEDKDGVEIINLEDKEACEEQHITVESRPLSQPQCKLIDEPEQLTLMDKSKVEEKNLSIQEQLIGTIGRVNVVPRRDNHKKKMAKIEEAELQKQKHVDKEED

SEQ ID NO: 6 - protein, 22 aa, Homo sapiens lymphocytic leukemia
CARDRRGEWPPSDYYYYYMDVW

SEQ ID NO: 7 - DNA, 70 bp, synthetic construct
  source 1..70: mol_type = other DNA
cggcgtaaacgccttatccggcccaggttttgctatctatctcctgagtcattgcttttcttttttcaca

SEQ ID NO: 8 - DNA, 70 bp, synthetic construct
  source 1..70: mol_type = other DNA
aaatgggcacggaaatccgtgccccaaaagagaaatggtatatctctgatgtaaagtgaatgataacgta

SEQ ID NO: 9 - DNA, 70 bp, synthetic construct
  source 1..70: mol_type = other DNA
ctggctcaaccgttattgctgaatttgaatcgctgggtcagtgcattcaccaccacaagcagataataac

SEQ ID NO: 10 - DNA, 70 bp, synthetic construct
  source 1..70: mol_type = other DNA
attgcggttattttaataaaattaagggttactattgagtcatagaacttccattattctcctgaagata

SEQ ID NO: 11 - DNA, 73 bp, synthetic construct
  source 1..73: mol_type = other DNA
actccgtgccgccggactgcgtgatgttattctccttactgcggcccatatccacctcaaccggatcgaaggc

SEQ ID NO: 12 - DNA, 88 bp, synthetic construct
  source 1..88: mol_type = other DNA
cgctttttatcgcaactctctactgtttctccatacccgtttttttggataggaggatgaaacgatgacgagcaaagaaacctttacc

SEQ ID NO: 13 - DNA, 72 bp, synthetic construct
  source 1..72: mol_type = other DNA
tgagtatagcctggtttcgtttgattggctgtggttttatacagtcattaaacgatgctgattgccgttccg

SEQ ID NO: 14 - DNA, 70 bp, synthetic construct
  source 1..70: mol_type = other DNA
cagccaatcaaacgaaaccaggctatactcaagcctggttttttgatggagttccggatctgcatcgcag

SEQ ID NO: 15 - DNA, 74 bp, synthetic construct
  source 1..74: mol_type = other DNA
tgcagaatccctgcttcgtccatttgacaggcacattatgcaagcattgctgtgataaactaccgcattaaagc

SEQ ID NO: 16 - DNA, 70 bp, synthetic construct
  source 1..70: mol_type = other DNA
gccgcacaggcggcctttagtgatgaagggtaaagcccttacactggtgtgttcagcaaatcgttaacgg

SEQ ID NO: 17 - DNA, 74 bp, synthetic construct
  source 1..74: mol_type = other DNA
cgcaactctctactgtttctccatacccgtttttttggaatgactgtataaaaccacagccaatcaaacgaaac

SEQ ID NO: 18 - protein, 138 aa, synthetic construct
MCARDRRGEWPPSDYYYYYMDVWGGGGSMTSKETFTHYQPQGNSDPAHTATAPGGLSAKAPAMTPLMLDTSSRKLVAWDGTTDGAAVGILAVAADQTSTTLTFYKSGTFRYEDVLWPEAASDETKKRTAFAGTAISIV

SEQ ID NO: 19 - protein, 258 aa, synthetic construct
MTSKETFTHYQPQGNSDPAHTATAPGGLSAKAPAMTPLMLDTSSRKLVAWDGTTDGAAVGILAVAADQTSTTLTFYKSGTFRYEDVLWPEAASDETKKRTAFAGTAISIVGGGGSASKSKEHKSKGKKDKGKKDKGKHKKAKKEKVKKHVVKNVIEDEDKDGVEIINLEDKEACEEQHITVESRPLSQPQCKLIDEPEQLTLMDKSKVEEKNLSIQEQLIGTIGRVNVVPRRDNHKKKMAKIEEAELQKQKHVDKEED

SEQ ID NO: 20 - protein, 310 aa, synthetic construct
MTSKETFTHYQPQGNSDPAHTATAPGGLSAKAPAMTPLMLDTSSRKLVAWDGTTDGAAVGILAVAADQTSTTLTFYKSGTFRYEDVLWPEAASDETKKRTAFAGTAISIVGGGGSGGGGSGGGGSDEYKDGVEIINLEDKEACEEQHITVESRPLSQPQCKLIDEPEQLTLMDKSKVEEKNLSIQEQLIGTIGRVNVVPRRDNHKKKMAKIEEAELQKQKHVDKEEDKKEESKEVEEESKEVQEDEEEVEEDEEEEEEEEEEEEEEEEEEEEEEGEVEEDEDDAEEDEEDEEEEEEEKKIKRNLRKNAKI

SEQ ID NO: 21 - protein, 301 aa, synthetic construct
MDEYKDGVEIINLEDKEACEEQHITVESRPLSQPQCKLIDEPEQLTLMDKSKVEEKNLSIQEQLIGTIGRVNVVPRRDNHKKKMAKIEEAELQKQKHVDKEEDKKEESKEVEEESKEVQEDEEEVEEDEEEEEEEEEEEEEEEEEEEEEEGEVEEDEDDAEEDEEDEEEEEEEKKIKRNLRKNAKIGGGGSMTSKETFTHYQPQGNSDPAHTATAPGGLSAKAPAMTPLMLDTSSRKLVAWDGTTDGAAVGILAVAADQTSTTLTFYKSGTFRYEDVLWPEAASDETKKRTAFAGTAISIV

SEQ ID NO: 22 - protein, 50 aa, synthetic construct
DLFMRIFTIGTVTLKQGEIKDATPSDFVRATATIPIQASLPFGWLIVGVA

SEQ ID NO: 23 - protein, 62 aa, synthetic construct
SDNGPQNQRNAPRITFGGPSDSTGSNQNGERSGARSKQRRPQGLPNNTASWFTALTQHGKED

SEQ ID NO: 24 - protein, 23 aa, synthetic construct
GALNTPKDHIGTRNPANNAAIVL

SEQ ID NO: 25 - protein, 47 aa, synthetic construct
TNTSNQVAVLYQDVNCTEVPVAIHADQLTPTWRVYSTGSNVFQTRAG

SEQ ID NO: 26 - protein, 24 aa, synthetic construct
SSSGWTAGAAAYYVGYLQPRTFLL

SEQ ID NO: 27 - protein, 133 aa, synthetic construct
FLLTTKRTMFVFLVLLPLVSSQCVNLTTRTQLPPAYTNSFTRGVYYPDKVFRSSVLHSTQDLFLPFFSNVTWFHAIHVSGTNGTKRFDNPVLPFNDGVYFASTEKSNIIRGWIFGTTLDSKTQSLLIVNNATN

SEQ ID NO: 28 - protein, 133 aa, synthetic construct
NATNVVIKVCEFQFCNDPFLGVYYHKNNKSWMESEFRVYSSANNCTFEYVSQPFLMDLEGKQGNFKNLREFVFKNIDGYFKIYSKHTPINLVRDLPQGFSALEPLVDLPIGINITRFQTLLALHRSYLTPGDS

SEQ ID NO: 29 - protein, 133 aa, synthetic construct
DSSSGWTAGAAAYYVGYLQPRTFLLKYNENGTITDAVDCALDPLSETKCTLKSFTVEKGIYQTSNFRVQPTESIVRFPNITNLCPFGEVFNATRFASVYAWNRKRISNCVADYSVLYNSASFSTFKCYGVSPT

SEQ ID NO: 30 - protein, 133 aa, synthetic construct
PTKLNDLCFTNVYADSFVIRGDEVRQIAPGQTGKIADYNYKLPDDFTGCVIAWNSNNLDSKVGGNYNYLYRLFRKSNLKPFERDISTEIYQAGSTPCNGVEGFNCYFPLQSYGFQPTNGVGYQPYRVVVLSFE

SEQ ID NO: 31 - protein, 133 aa, synthetic construct
FELLHAPATVCGPKKSTNLVKNKCVNFNFNGLTGTGVLTESNKKFLPFQQFGRDIADTTDAVRDPQTLEILDITPCSFGGVSVITPGTNTSNQVAVLYQDVNCTEVPVAIHADQLTPTWRVYSTGSNVFQTRA

SEQ ID NO: 32 - protein, 133 aa, synthetic construct
RAGCLIGAEHVNNSYECDIPIGAGICASYQTQTNSPRRARSVASQSIIAYTMSLGAENSVAYSNNSIAIPTNFTISVTTEILPVSMTKTSVDCTMYICGDSTECSNLLLQYGSFCTQLNRALTGIAVEQDKNT

SEQ ID NO: 33 - protein, 133 aa, synthetic construct
NTQEVFAQVKQIYKTPPIKDFGGFNFSQILPDPSKPSKRSFIEDLLFNKVTLADAGFIKQYGDCLGDIAARDLICAQKFNGLTVLPPLLTDEMIAQYTSALLAGTITSGWTFGAGAALQIPFAMQMAYRFNGI

SEQ ID NO: 34 - protein, 133 aa, synthetic construct
NGIGVTQNVLYENQKLIANQFNSAIGKIQDSLSSTASALGKLQDVVNQNAQALNTLVKQLSSNFGAISSVLNDILSRLDKVEAEVQIDRLITGRLQSLQTYVTQQLIRAAEIRASANLAATKMSECVLGQSKR

SEQ ID NO: 35 - protein, 75 aa, synthetic construct
MYSFVSEETGTLIVNSVLLFLAFVVFLLVTLAILTALRLCAYCCNIVNVSLVKPSFYVYSRVKNLNSSRVPDLLV

SEQ ID NO: 36 - protein, 401 aa, bacteriophage lambda
MAVKISGVLKDGTGKPVQNCTIQLKARRNSTTVVVNTVGSENPDEAGRYSMDVEYGQYSVILQVDGFPPSHAGTITVYEDSQPGTLNDFLCAMTEDDARPEVLRRLELMVEEVARNASVVAQSTADAKKSAGDASASAAQVAALVTDATDSARAASTSAGQAASSAQEASSGAEAASAKATEAEKSAAAAESSKNAAATSAGAAKTSETNAAASQQSAATSASTAATKASEAATSARDAVASKEAAKSSETNASSSAGRAASSATAAENSARAAKTSETNARSSETAAERSASAAADAKTAAAGSASTASTKATEAAGSAVSASQSKSAAEAAAIRAKNSAKRAEDIASAVALEDADTTRKGIVQLSSATNSTSETLAATPKAVKVVMDETNRKAHWTVRH

SEQ ID NO: 37 - protein, 246 aa, bacteriophage lambda
MPVPNPTMPVKGAGTTLWVYKGSGDPYANPLSDVDWSRLAKVKDLTPGELTAESYDDSYLDDEDADWTATGQGQKSAGDTSFTLAWMPGEQGQQALLAWFNEGDTRAYKIRFPNGTVDVFRGWVSSIGKAVTAKEVITRTVKVTNVGRPSMAEDRSTVTAATGMTVTPASTSVVKGQSTTLTVAFQPEGVTDKSFRAVSADKTKATVSVSGMTITVNGVAAGKVNIPVVSGNGEFAAVAEITVTAS

SEQ ID NO: 38 - protein, 23 aa, Severe acute respiratory syndrome-related coronavirus
FKEELDKYFKNHTSPDVDLGDIS

SEQ ID NO: 39 - protein, 108 aa, synthetic construct
LGDISGINASVVNIQKEIDRLNEVAKNLNESLIDLQELGKYEQYIKWPWYIWLGFIAGLIAIVMVTIMLCCMTSCCSCLKGCCSCGSCCKFDEDDSEPVLKGVKLHYT

SEQ ID NO: 40 - protein, 33 aa, Severe acute respiratory syndrome-related coronavirus
KRVDFCGKGYHLMSFPQSAPHGVVFLHVTYVPA

SEQ ID NO: 41 - protein, 33 aa, Severe acute respiratory syndrome-related coronavirus
VVFLHVTYVPAQEKNFTTAPAICHDGKAHFPRE

SEQ ID NO: 42 - protein, 33 aa, Severe acute respiratory syndrome-related coronavirus
CHDGKAHFPREGVFVSNGTHWFVTQRNFYEPQI

SEQ ID NO: 43 - protein, 33 aa, Severe acute respiratory syndrome-related coronavirus
VTQRNFYEPQIITTDNTFVSGNCDVVIGIVNNT

SEQ ID NO: 44 - protein, 33 aa, Severe acute respiratory syndrome-related coronavirus
CDVVIGIVNNTVYDPLQPELDSFKEELDKYFKN

SEQ ID NO: 45 - protein, 23 aa, Severe acute respiratory syndrome-related coronavirus
FKEELDKYFKNHTSPDVDLGDIS

SEQ ID NO: 46 - protein, 84 aa, Severe acute respiratory syndrome-related coronavirus
MSFPQSAPHGVVFLHVTYVPAQEKNFTTAPAICHDGKAHFPREGVFVSNGTHWFVTQRNFYEPQIITTDNTFVSGNCDVVIGIV

SEQ ID NO: 47 - protein, 31 aa, Severe acute respiratory syndrome-related coronavirus
YDPLQPELDSFKEELDKYFKNHTSPDVDLGD

SEQ ID NO: 48 - protein, 30 aa, Severe acute respiratory syndrome-related coronavirus
GGFNFSQILPDPSKPSKRSFIEDLLFNKVT

SEQ ID NO: 49 - protein, 30 aa, Severe acute respiratory syndrome-related coronavirus
CDIPIGAGICASYQTQTNSPRRARSVASQS

SEQ ID NO: 50 - protein, 30 aa, Severe acute respiratory syndrome-related coronavirus
NNLDSKVGGNYNYLYRLFRKSNLKPFERDI

SEQ ID NO: 51 - protein, 30 aa, Severe acute respiratory syndrome-related coronavirus
NLKPFERDISTEIYQAGSTPCNGVEGFNCY

SEQ ID NO: 52 - protein, 30 aa, Severe acute respiratory syndrome-related coronavirus
NGVEGFNCYFPLQSYGFQPTNGVGYQPYRV

SEQ ID NO: 53 - protein, 13 aa, synthetic construct
LEEKKGNYVVTDH

SEQ ID NO: 54 - protein, 13 aa, synthetic construct
LEEKKYNYVVTDH

SEQ ID NO: 55-56 - skipped (2 entries)

SEQ ID NO: 57 - DNA, 1871 bp, synthetic construct
  source 1..1871: mol_type = other DNA
cgcaatgcttgcataatgtgcctgtcaaatggacgaagcagggattctgcaaaccctatgctactccgtcaagccgtcaattgtctgattcgttaccaattatgacaacttgacggctacatcattcactttttcttcacaaccggcacgaaactcgctcgggctggccccggtgcattttttaaatactcgcgagaaatagagttgatcgtcaaaaccaacattgcgaccgacggtggcgataggcatccgggtagtgctcaaaagcagcttcgcctgactaatgcgttggtcctcgcgccagcttaagacgctaatccctaactgctggcggaaaagatgtgacagacgcgacggcgacaagcaaacatgctgtgcgacgctggcgatatcaaaattgctgtctgccaggtgatcgctgatgtactgacaagcctcgcgtacccgattatccatcggtggatggagcgactcgttaatcgcttccatgcgccgcagtaacaattgctcaagcagatttatcgccagcagctccgaatagcgcccttccccttgcccggcgttaatgatttgcccaaacaggtcgctgaaatgcggctggtgcgcttcatccgggcgaaagaaacccgtattggcaaatattgacggccagttaagccattcatgccagtaggcgcgcggacgaaagtaaacccactggtgataccattcgcgagcctccggatgacgaccgtagtgatgaatctctcctggcgggaacagcaaaatatcacccggtcggcagacaaattctcgtccctgatttttcaccaccccctgaccgcgaatggtgagattgagaatataacctttcattcccagcggtcggtcgataaaaaaatcgagataaccgttggcctcaatcggcgttaaacccgccaccagatgggcgttaaacgagtatcccggcagcaggggatcattttgcgcttcagccatacttttcatactcccaccattcagagaagaaaccaattgtccatattgcatcagacattgccgtcactgcgtcttttactggctcttctcgctaacccaaccggtaaccccgcttattaaaagcattctgtaacaaagcgggaccaaagccatgacaaaaacgcgtaacaaaagtgtctataatcacggcagaaaagtccacattgattatttgcacggcgtcacactttgctatgccatagcatttttatccataagattagcggatcctacctgacgctttttatcgcaactctctactgtttctccatacccgtttttttggataggaggatgaaacgatgacgagcaaagaaacctttacccattaccagccgcagggcaacagtgacccggctcataccgcaaccgcgcccggcggattgagtgcgaaagcgcctgcaatgaccccgctgatgctggacacctccagccgtaagctggttgcgtgggatggcaccaccgacggtgctgccgttggcattcttgcggttgctgctgaccagaccagcaccacgctgacgttctacaagtccggcacgttccgttatgaggatgtgctctggccggaggctgccagcgacgagacgaaaaaacggaccgcgtttgccggaacggcaatcagcatcgtttaatgactgtataaaaccacagccaatcaaacgaaaccaggctatactcaagcctggttttttgatggaattacagcgtggcgcaggcaggttttatcttaacccgacactggcgggacaccccgcaagggacagaagtctccttctggctggcgacggacaacgggcctcagttgctcaatgtacctataaccagaccgttcagctggatattacggcctt

SEQ ID NO: 58 - DNA, 285 bp, synthetic construct
  source 1..285: mol_type = other DNA
aagaaaccaattgtccatattgcatcagacattgccgtcactgcgtcttttactggctcttctcgctaacccaaccggtaaccccgcttattaaaagcattctgtaacaaagcgggaccaaagccatgacaaaaacgcgtaacaaaagtgtctataatcacggcagaaaagtccacattgattatttgcacggcgtcacactttgctatgccatagcatttttatccataagattagcggatcctacctgacgctttttatcgcaactctctactgtttctccat

SEQ ID NO: 59 - DNA, 30 bp, synthetic construct
  source 1..30: mol_type = other DNA
acccgtttttttggataggaggatgaaacg

SEQ ID NO: 60 - protein, 292 aa, synthetic construct
MAEAQNDPLLPGYSFNAHLVAGLTPIEANGYLDFFIDRPLGMKGYILNLTIRGQGVVKNQGREFVCRPGDILLFPPGEIHHYGRHPEAREWYHQWVYFRPRAYWHEWLNWPSIFANTGFFRPDEAHQPHFSDLFGQIINAGQGEGRYSELLAINLLEQLLLRRMEAINESLHPPMDNRVREACQYISDHLADSNFDIASVAQHVCLSPSRLSHLFRQQLGISVLSWREDQRISQAKLLLSTTRMPIATVGRNVGFDDQLYFSRVFKKCTGASPSEFRAGCEEKVNDVAVKLS

SEQ ID NO: 61 - protein, 783 aa, synthetic construct
MAQAGFILTRHWRDTPQGTEVSFWLATDNGPLQVTLAPQESVAFIPADQVPRAQHILQGEQGFRLTPLALKDFHRQPVYGLYCRAHRQLMNYEKRLREGGVTVYEADVRPPERYLMERFITSPVWVEGDMHNGTIVNARLKPHPDYRPPLKWVSIDIETTRHGELYCIGLEGCGQRIVYMLGPENGDASSLDFELEYVASRPQLLEKLNAWFANYDPDVIIGWNVVQFDLRMLQKHAERYRLPLRLGRDNSELEWREHGFKNGVFFAQAKGRLIIDGIEALKSAFWNFSSFSLETVAQELLGEGKSIDNPWDRMDEIDRRFAEDKPALATYNLKDCELVTQIFHKTEIMPFLLERATVNGLPVDRHGGSVAAFGHLYFPRMHRAGYVAPNLGEVPPHASPGGYVMDSRPGLYDSVLVLDYKSLYPSIIRTFLIDPVGLVEGMAQPDPEHSTEGFLDAWFSREKHCLPEIVTNIWHGRDEAKRQGNKPLSQALKIIMNAFYGVLGTTACRFFDPRLASSITMRGHQIMRQTKALIEAQGYDVIYGDTDSTFVWLKGAHSEEEAAKIGRALVQHVNAWWAETLQKQRLTSALELEYETHFCRFLMPTIRGADTGSKKRYAGLIQEGDKQRMVFKGLETVRTDWTPLAQQFQQELYLRIFRNEPYQEYVRETIDKLMAGELDARLVYRKRLRRPLSEYQRNVPPHVRAARLADEENQKRGRPLQYQNRGTIKYVWTTNGPEPLDYQRSPLDYEHYLTRQLQPVAEGILPFIEDNFATLMTGQLGLF

SEQ ID NO: 62 - DNA, 4471 bp, synthetic construct
  source 1..4471: mol_type = other DNA
cgtttttttggataggaggatgaaacgatgacgagcaaagaaacctttacccattaccagccgcagggcaacagtgacccggctcataccgcaaccgcgcccggcggattgagtgcgaaagcgcctgcaatgaccccgctgatgctggacacctccagccgtaagctggttgcgtgggatggcaccaccgacggtgctgccgttggcattcttgcggttgctgctgaccagaccagcaccacgctgacgttctacaagtccggcacgttccgttatgaggatgtgctctggccggaggctgccagcgacgagacgaaaaaacggaccgcgtttgccggaacggcaatcagcatcgtttaatgactgtataaaaccacagccaatcaaacgaaaccaggctatactcaagcctggttttttgatggagttccggatctgcatcgcaggatgctgctggctaccctgtggaacacctacatctgtattaacgaagcgctggcattgaccctgagtgatttttctctggtcccgccgcatccataccgccagttgtttaccctcacaacgttccagtaaccgggcatgttcatcatcagtaacccgtatcgtgagcatcctctctcgtttcatcggtatcattacccccatgaacagaaatcccccttacacggaggcatcagtgaccaaacaggaaaaaaccgcccttaacatggcccgctttatcagaagccagacattaacgcttctggagaaactcaacgagctggacgcggatgaacaggcagacatctgtgaatcgcttcacgaccacgctgatgagctttaccgcagctgcctcgcgcgtttcggtgatgacggtgaaaacctctgacacatgcagctcccggagacggtcacagcttgtctgtaagcggatgccgggagcagacaagcccgtcagggcgcgtcagcgggtgttggcgggtgtcggggcgcagccatgacccagtcacgtagcgatagcggagtgtatactggcttaactatgcggcatcagagcagattgtactgagagtgcaccatatgcggtgtgaaataccgcacagatgcgtaaggagaaaataccgcatcaggcgctcttccgcttcctcgctcactgactcgctgcgctcggtcgttcggctgcggcgagcggtatcagctcactcaaaggcggtaatacggttatccacagaatcaggggataacgcaggaaagaacatgtgagcaaaaggccagcaaaaggccaggaaccgtaaaaaggccgcgttgctggcgtttttccataggctccgcccccctgacgagcatcacaaaaatcgacgctcaagtcagaggtggcgaaacccgacaggactataaagataccaggcgtttccccctggaagctccctcgtgcgctctcctgttccgaccctgccgcttaccggatacctgtccgcctttctcccttcgggaagcgtggcgctttctcatagctcacgctgtaggtatctcagttcggtgtaggtcgttcgctccaagctgggctgtgtgcacgaaccccccgttcagcccgaccgctgcgccttatccggtaactatcgtcttgagtccaacccggtaagacacgacttatcgccactggcagcagccactggtaacaggattagcagagcgaggtatgtaggcggtgctacagagttcttgaagtggtggcctaactacggctacactagaaggacagtatttggtatctgcgctctgctgaagccagttaccttcggaaaaagagttggtagctcttgatccggcaaacaaaccaccgctggtagcggtggtttttttgtttgcaagcagcagattacgcgcagaaaaaaaggatctcaagaagatcctttgatcttttctacggggtctgacgctcagtggaacgaaaactcacgttaagggattttggtcatgagattatcaaaaaggatcttcacctagatccttttaaattaaaaatgaagttttaaatcaatctaaagtatatatgagtaaacttggtctgacagttaccaatgcttaatcagtgaggcacctatctcagcgatctgtctatttcgttcatccatagttgcctgactccccgtcgtgtagataactacgatacgggagggcttaccatctggccccagtgctgcaatgataccgcgagacccacgctcaccggctccagatttatcagcaataaaccagccagccggaagggccgagcgcagaagtggtcctgcaactttatccgcctccatccagtctattaattgttgccgggaagctagagtaagtagttcgccagttaatagtttgcgcaacgttgttgccattgctgcaggcatcgtggtgtcacgctcgtcgtttggtatggcttcattcagctccggttcccaacgatcaaggcgagttacatgatcccccatgttgtgcaaaaaagcggttagctccttcggtcctccgatcgttgtcagaagtaagttggccgcagtgttatcactcatggttatggcagcactgcataattctcttactgtcatgccatccgtaagatgcttttctgtgactggtgagtactcaaccaagtcattctgagaatagtgtatgcggcgaccgagttgctcttgcccggcgtcaacacgggataataccgcgccacatagcagaactttaaaagtgctcatcattggaaaacgttcttcggggcgaaaactctcaaggatcttaccgctgttgagatccagttcgatgtaacccactcgtgcacccaactgatcttcagcatcttttactttcaccagcgtttctgggtgagcaaaaacaggaaggcaaaatgccgcaaaaaagggaataagggcgacacggaaatgttgaatactcatactcttcctttttcaatattattgaagcatttatcagggttattgtctcatgagcggatacatatttgaatgtatttagaaaaataaacaaataggggttccgcgcacatttccccgaaaagtgccacctgacgtctaagaaaccattattatcatgacattaacctataaaaataggcgtatcacgaggccctttcgtcttcaagaattctcatgtttgacagcttatcatcgataagctttaatgcggtagtttatcacagcaatgcttgcataatgtgcctgtcaaatggacgaagcagggattctgcaaaccctatgctactccgtcaagccgtcaattgtctgattcgttaccaattatgacaacttgacggctacatcattcactttttcttcacaaccggcacgaaactcgctcgggctggccccggtgcattttttaaatactcgcgagaaatagagttgatcgtcaaaaccaacattgcgaccgacggtggcgataggcatccgggtagtgctcaaaagcagcttcgcctgactaatgcgttggtcctcgcgccagcttaagacgctaatccctaactgctggcggaaaagatgtgacagacgcgacggcgacaagcaaacatgctgtgcgacgctggcgatatcaaaattgctgtctgccaggtgatcgctgatgtactgacaagcctcgcgtacccgattatccatcggtggatggagcgactcgttaatcgcttccatgcgccgcagtaacaattgctcaagcagatttatcgccagcagctccgaatagcgcccttccccttgcccggcgttaatgatttgcccaaacaggtcgctgaaatgcggctggtgcgcttcatccgggcgaaagaaacccgtattggcaaatattgacggccagttaagccattcatgccagtaggcgcgcggacgaaagtaaacccactggtgataccattcgcgagcctccggatgacgaccgtagtgatgaatctctcctggcgggaacagcaaaatatcacccggtcggcagacaaattctcgtccctgatttttcaccaccccctgaccgcgaatggtgagattgagaatataacctttcattcccagcggtcggtcgataaaaaaatcgagataaccgttggcctcaatcggcgttaaacccgccaccagatgggcgttaaacgagtatcccggcagcaggggatcattttgcgcttcagccatacttttcatactcccaccattcagagaagaaaccaattgtccatattgcatcagacattgccgtcactgcgtcttttactggctcttctcgctaacccaaccggtaaccccgcttattaaaagcattctgtaacaaagcgggaccaaagccatgacaaaaacgcgtaacaaaagtgtctataatcacggcagaaaagtccacattgattatttgcacggcgtcacactttgctatgccatagcatttttatccataagattagcggatcctacctgacgctttttatcgcaactctctactgtttctccatacc

SEQ ID NO: 63 - protein, 589 aa, synthetic construct
TTTCCATAGGCTCCGCCCCCCTGACGAGCATCACAAAAATCGACGCTCAAGTCAGAGGTGGCGAAACCCGACAGGACTATAAAGATACCAGGCGTTTCCCCCTGGAAGCTCCCTCGTGCGCTCTCCTGTTCCGACCCTGCCGCTTACCGGATACCTGTCCGCCTTTCTCCCTTCGGGAAGCGTGGCGCTTTCTCATAGCTCACGCTGTAGGTATCTCAGTTCGGTGTAGGTCGTTCGCTCCAAGCTGGGCTGTGTGCACGAACCCCCCGTTCAGCCCGACCGCTGCGCCTTATCCGGTAACTATCGTCTTGAGTCCAACCCGGTAAGACACGACTTATCGCCACTGGCAGCAGCCACTGGTAACAGGATTAGCAGAGCGAGGTATGTAGGCGGTGCTACAGAGTTCTTGAAGTGGTGGCCTAACTACGGCTACACTAGAAGGACAGTATTTGGTATCTGCGCTCTGCTGAAGCCAGTTACCTTCGGAAAAAGAGTTGGTAGCTCTTGATCCGGCAAACAAACCACCGCTGGTAGCGGTGGTTTTTTTGTTTGCAAGCAGCAGATTACGCGCAGAAAAAAAGGATCTCAA

SEQ ID NO: 64 - protein, 286 aa, synthetic construct [sequence omitted]

SEQ ID NO: 65 - DNA, 88 bp, synthetic construct; identical to SEQ ID NO: 12
  source 1..88: mol_type = other DNA

SEQ ID NO: 66 - DNA, 72 bp, synthetic construct; identical to SEQ ID NO: 13
  source 1..72: mol_type = other DNA

SEQ ID NO: 67 - DNA, 70 bp, synthetic construct; identical to SEQ ID NO: 14
  source 1..70: mol_type = other DNA

SEQ ID NO: 68 - DNA, 74 bp, synthetic construct; identical to SEQ ID NO: 15
  source 1..74: mol_type = other DNA

SEQ ID NO: 69 - protein, 11 aa, Severe acute respiratory syndrome-related coronavirus
FKEELDKYFKN